European Patent Specification EP 2 940 029 B1, published November 29, 2023. Title: Design and Synthesis of Cleavable Fluorescent Nucleotides as Reversible Terminators for DNA Sequencing by Synthesis. Applicant: The Trustees of Columbia University in the City of New York. The sequence listing filed with the application follows.

SEQUENCE LISTING (17 sequences)

SEQ ID NO: 1 - DNA, 26 bp, Artificial Sequence
  self-priming DNA template for Polymerase extension reaction
atcggcgccgcgccttggcgcggcgc

SEQ ID NO: 2 - DNA, 26 bp, Artificial Sequence
  self-priming DNA template for polymerase extension reaction
gactgcgccgcgccttggcgcggcgc

SEQ ID NO: 3 - DNA, 26 bp, Artificial Sequence
  self-priming DNA template for polymerase extension reaction
atcggcgccgcgccttggcgcggcgc

SEQ ID NO: 4 - DNA, 26 bp, Artificial Sequence
  self-priming DNA template for polymerase extension reaction for ddGTP-N3-Cy5
gatcgcgccgcgccttggcgcggcgc

SEQ ID NO: 5 - DNA, 26 bp, Artificial Sequence
  self-priming DNA template for polymerase extension reaction for ddNTP-N3-R6G
gtcagcgccgcgccttggcgcggcgc

SEQ ID NO: 6 - DNA, 80 bp, Artificial Sequence
  5' -amino-labeled self-priming DNA template for polymerase extension reaction
cactcacatatgttttttagcttttttaatttcttaatgatgttgttgcatgcgacttaaggcgcttgcgccttaagtcg

SEQ ID NO: 7 - DNA, 15 bp, Artificial Sequence
  15 nucleotides of a 130 bp self-priming DNA template for polymerase extension reaction
actgaacatctgcat

SEQ ID NO: 8 - DNA, 21 bp, Artificial Sequence
  21 nucleotides of a self-priming DNA template for polymerase extension reaction
tgttaatcatgttgttgcatg

SEQ ID NO: 9 - DNA, 14 bp, Artificial Sequence
  DNA template for template "walking"
aatcatctcgcatg

SEQ ID NO: 10 - DNA, 10 bp, Artificial Sequence
  Polymerase extension reaction product of SEQ ID No: 9
  modified_base (10)..(10): R6G-R2
catgcgagau

SEQ ID NO: 11 - DNA, 10 bp, Artificial Sequence
  Polymerase extension reaction product of SEQ ID No: 9
  modified_base (10)..(10): 3'-R1
catgcgagat

SEQ ID NO: 12 - DNA, 14 bp, Artificial Sequence
  DNA template for template "walking"
aatctactagcatg

SEQ ID NO: 13 - DNA, 10 bp, Artificial Sequence
  Polymerase extension reaction product of SEQ ID No: 12
  modified_base (10)..(10): ROX-R2
catgctagta

SEQ ID NO: 14 - DNA, 10 bp, Artificial Sequence
  Polymerase extension reaction product of SEQ ID No: 12
  modified_base (10)..(10): 3'-R1
catgctagta

SEQ ID NO: 15 - DNA, 10 bp, Artificial Sequence
  Polymerase extension reaction product of SEQ ID No: 9
  modified_base (10)..(10): R6G-R2; 3'-R1
catgcgagau

SEQ ID NO: 16 - DNA, 10 bp, Artificial Sequence
  Polymerase extension reaction product of SEQ ID No: 12
  modified_base (10)..(10): ROX-R2; 3'-R1
catgctagta

SEQ ID NO: 17 - DNA, 10 bp, Artificial Sequence
  Polymerase extension reaction product of SEQ ID No: 12
  modified_base (10)..(10): 3'-R1
catgctagua